European Patent Specification EP 3 656 792 B1, published July 3, 2024. Title: IMMUNOGLOBULIN Fc VARIANTS. Applicant: HANMI SCIENCE CO., LTD. The sequence listing filed with the application follows.

SEQUENCE LISTING (119 sequences)

SEQ ID NO: 1 - DNA, 34 bp, Artificial Sequence
  primer FcM202Lss
cttctcatgctccgtgctgcatgaggctctgcac

SEQ ID NO: 2 - DNA, 34 bp, Artificial Sequence
  primer FcM202Las
gtgcagagcctcatgcagcacggagcatgagaag

SEQ ID NO: 3 - DNA, 33 bp, Artificial Sequence
  primer FcN208Sss
catgaggctctgcacagccactacacacagaag

SEQ ID NO: 4 - DNA, 33 bp, Artificial Sequence
  primer FcN208Sas
cttctgtgtgtagtggctgtgcagagcctcatg

SEQ ID NO: 5 - DNA, 34 bp, Artificial Sequence
  primer FcI27Fss
caaggacaccctcatgttctcccggacccctgag

SEQ ID NO: 6 - DNA, 34 bp, Artificial Sequence
  primer FcI27Fas
ctcaggggtccgggagaacatgagggtgtccttg

SEQ ID NO: 7 - DNA, 34 bp, Artificial Sequence
  primer FcH207Tss
gatgcatgaggctctgaccaaccactacacacag

SEQ ID NO: 8 - DNA, 34 bp, Artificial Sequence
  primer FcH207Tas
ctgtgtgtagtggttggtcagagcctcatgcatc

SEQ ID NO: 9 - DNA, 34 bp, Artificial Sequence
  primer FcH207Kss
gatgcatgaggctctgaagaaccactacacacag

SEQ ID NO: 10 - DNA, 34 bp, Artificial Sequence
  primer FcH207Kas
ctgtgtgtagtggttcttcagagcctcatgcatc

SEQ ID NO: 11 - DNA, 34 bp, Artificial Sequence
  primer FcL83Fss
cagcgtcctcaccgtcttccaccaggactggctg

SEQ ID NO: 12 - DNA, 34 bp, Artificial Sequence
  primer FcL83Fas
cagccagtcctggtggaagacggtgaggacgctg

SEQ ID NO: 13 - DNA, 34 bp, Artificial Sequence
  primer FcI27Lss
caaggacaccctcatgctctcccggacccctgag

SEQ ID NO: 14 - DNA, 34 bp, Artificial Sequence
  primer FcI27Las
ctcaggggtccgggagagcatgagggtgtccttg

SEQ ID NO: 15 - DNA, 34 bp, Artificial Sequence
  primer FcH207K/N208Sss
gatgcatgaggctctgaagagccactacacacag

SEQ ID NO: 16 - DNA, 34 bp, Artificial Sequence
  primer FcH207K/N208Sas
ctgtgtgtagtggctcttcagagcctcatgcatc

SEQ ID NO: 17 - DNA, 33 bp, Artificial Sequence
  primer FcN208Tss
catgaggctctgcacacccactacacacagaag

SEQ ID NO: 18 - DNA, 33 bp, Artificial Sequence
  primer FcN208Tas
cttctgtgtgtagtgggtgtgcagagcctcatg

SEQ ID NO: 19 - DNA, 34 bp, Artificial Sequence
  primer FcH207T/N208Sss
gatgcatgaggctctgaccagccactacacacag

SEQ ID NO: 20 - DNA, 34 bp, Artificial Sequence
  primer FcH207T/N208Sas
ctgtgtgtagtggctggtcagagcctcatgcatc

SEQ ID NO: 21 - DNA, 34 bp, Artificial Sequence
  primer FcE204Rss
atgctccgtgatgcatcgggctctgcacaaccac

SEQ ID NO: 22 - DNA, 34 bp, Artificial Sequence
  primer FcE204Ras
gtggttgtgcagagcccgatgcatcacggagcat

SEQ ID NO: 23 - DNA, 34 bp, Artificial Sequence
  primer FcE204Kss
atgctccgtgatgcataaggctctgcacaaccac

SEQ ID NO: 24 - DNA, 34 bp, Artificial Sequence
  primer FcE204Kas
gtggttgtgcagagccttatgcatcacggagcat

SEQ ID NO: 25 - DNA, 42 bp, Artificial Sequence
  primer FcE204R/H207Kss
tgctccgtgatgcatcgggctctgaagaaccactacacacag

SEQ ID NO: 26 - DNA, 42 bp, Artificial Sequence
  primer FcE204R/H207Kas
ctgtgtgtagtggttcttcagagcccgatgcatcacggagca

SEQ ID NO: 27 - DNA, 42 bp, Artificial Sequence
  primer FcE204K/H207Kss
tgctccgtgatgcataaggctctgaagaaccactacacacag

SEQ ID NO: 28 - DNA, 42 bp, Artificial Sequence
  primer FcE204K/H207Kas
ctgtgtgtagtggttcttcagagccttatgcatcacggagca

SEQ ID NO: 29 - DNA, 34 bp, Artificial Sequence
  primer FcH203Rss
ctcatgctccgtgatgcgtgaggctctgcacaac

SEQ ID NO: 30 - DNA, 34 bp, Artificial Sequence
  primer FcH203Ras
gttgtgcagagcctcacgcatcacggagcatgag

SEQ ID NO: 31 - DNA, 34 bp, Artificial Sequence
  primer FcH203Kss
ctcatgctccgtgatgaaggaggctctgcacaac

SEQ ID NO: 32 - DNA, 34 bp, Artificial Sequence
  primer FcH203Kas
gttgtgcagagcctccttcatcacggagcatgag

SEQ ID NO: 33 - DNA, 44 bp, Artificial Sequence
  primer FcH203R/H207Kss
catgctccgtgatgcgtgaggctctgaagaaccactacacacag

SEQ ID NO: 34 - DNA, 44 bp, Artificial Sequence
  primer FcH203R/H207Kas
ctgtgtgtagtggttcttcagagcctcacgcatcacggagcatg

SEQ ID NO: 35 - DNA, 44 bp, Artificial Sequence
  primer FcH203K/H207Kss
catgctccgtgatgaaggaggctctgaagaaccactacacacag

SEQ ID NO: 36 - DNA, 44 bp, Artificial Sequence
  primer FcH203K/H207Kas
ctgtgtgtagtggttcttcagagcctccttcatcacggagcatg

SEQ ID NO: 37 - DNA, 49 bp, Artificial Sequence
  primer FcM202L/H207Kss
cttctcatgctccgtgctgcatgaggctctgaagaaccactacacacag

SEQ ID NO: 38 - DNA, 49 bp, Artificial Sequence
  primer FcM202L/H207Kas
ctgtgtgtagtggttcttcagagcctcatgcagcacggagcatgagaag

SEQ ID NO: 39 - DNA, 49 bp, Artificial Sequence
  primer FcH203K/N208Tss
ctcatgctccgtgatgaaggaggctctgcacacccactacacacagaag

SEQ ID NO: 40 - DNA, 49 bp, Artificial Sequence
  primer FcH203K/N208Tas
cttctgtgtgtagtgggtgtgcagagcctccttcatcacggagcatgag

SEQ ID NO: 41 - DNA, 33 bp, Artificial Sequence
  primer FcT81Ess
gtggtcagcgtcctcgaagtcctgcaccaggac

SEQ ID NO: 42 - DNA, 33 bp, Artificial Sequence
  primer FcT81Eas
gtcctggtgcaggacttcgaggacgctgaccac

SEQ ID NO: 43 - DNA, 33 bp, Artificial Sequence
  primer FcE154Ass
agcgacatcgccgtggcgtgggagagcaatggg

SEQ ID NO: 44 - DNA, 33 bp, Artificial Sequence
  primer FcE154Aas
cccattgctctcccacgccacggcgatgtcgct

SEQ ID NO: 45 - DNA, 33 bp, Artificial Sequence
  primer FcE154Sss
agcgacatcgccgtgtcgtgggagagcaatggg

SEQ ID NO: 46 - DNA, 33 bp, Artificial Sequence
  primer FcE154Sas
cccattgctctcccacgacacggcgatgtcgct

SEQ ID NO: 47 - DNA, 33 bp, Artificial Sequence
  primer FcV82Pss
gtcagcgtcctcacccccctgcaccaggactgg

SEQ ID NO: 48 - DNA, 33 bp, Artificial Sequence
  primer FcV82Pas
ccagtcctggtgcaggggggtgaggacgctgac

SEQ ID NO: 49 - DNA, 33 bp, Artificial Sequence
  primer FcE204Sss
tgctccgtgatgcattcggctctgcacaaccac

SEQ ID NO: 50 - DNA, 33 bp, Artificial Sequence
  primer FcE204Sas
gtggttgtgcagagccgaatgcatcacggagca

SEQ ID NO: 51 - DNA, 33 bp, Artificial Sequence
  primer FcT81Sss
gtggtcagcgtcctctccgtcctgcaccaggac

SEQ ID NO: 52 - DNA, 33 bp, Artificial Sequence
  primer FcT81Sas
gtcctggtgcaggacggagaggacgctgaccac

SEQ ID NO: 53 - DNA, 34 bp, Artificial Sequence
  primer FcH203A/E204Sss
tcatgctccgtgatggcttcggctctgcacaacc

SEQ ID NO: 54 - DNA, 34 bp, Artificial Sequence
  primer FcH203A/E204Sas
ggttgtgcagagccgaagccatcacggagcatga

SEQ ID NO: 55 - DNA, 34 bp, Artificial Sequence
  primer FcH207A/N208Sss
gatgcatgaggctctggccagccactacacacag

SEQ ID NO: 56 - DNA, 34 bp, Artificial Sequence
  primer FcH207A/N208Sas
ctgtgtgtagtggctggccagagcctcatgcatc

SEQ ID NO: 57 - DNA, 32 bp, Artificial Sequence
  primer FcE204A/N208Sss
gctccgtgatgcatgcggctctgcacagccac

SEQ ID NO: 58 - DNA, 32 bp, Artificial Sequence
  primer FcE204A/N208Sas
gtggctgtgcagagccgcatgcatcacggagc

SEQ ID NO: 59 - DNA, 34 bp, Artificial Sequence
  primer FcH203A/N208Sss
ctcatgctccgtgatggctgaggctctgcacagc

SEQ ID NO: 60 - DNA, 34 bp, Artificial Sequence
  primer FcH203A/N208Sas
gctgtgcagagcctcagccatcacggagcatgag

SEQ ID NO: 61 - DNA, 34 bp, Artificial Sequence
  primer FcM202A/N208Sss
cttctcatgctccgtggcgcatgaggctctgcac

SEQ ID NO: 62 - DNA, 34 bp, Artificial Sequence
  primer FcM202A/N208Sas
gtgcagagcctcatgcgccacggagcatgagaag

SEQ ID NO: 63 - DNA, 34 bp, Artificial Sequence
  primer FcY93Lss
gctgaatggcaaggagctcaagtgcaaggtctcc

SEQ ID NO: 64 - DNA, 34 bp, Artificial Sequence
  primer FcY93Las
ggagaccttgcacttgagctccttgccattcagc

SEQ ID NO: 65 - DNA, 33 bp, Artificial Sequence
  primer FcV82Lss
ggtcagcgtcctcaccctcctgcaccaggactg

SEQ ID NO: 66 - DNA, 33 bp, Artificial Sequence
  primer FcV82Las
cagtcctggtgcaggagggtgaggacgctgacc

SEQ ID NO: 67 - DNA, 34 bp, Artificial Sequence
  primer FcT81Ass
gtgtggtcagcgtcctcgccgtcctgcaccagga

SEQ ID NO: 68 - DNA, 34 bp, Artificial Sequence
  primer FcT81Aas
tcctggtgcaggacggcgaggacgctgaccacac

SEQ ID NO: 69 - DNA, 34 bp, Artificial Sequence
  primer FcH207L/N208Sss
gatgcatgaggctctgctcagccactacacacag

SEQ ID NO: 70 - DNA, 34 bp, Artificial Sequence
  primer FcH207L/N208Sas
ctgtgtgtagtggctgagcagagcctcatgcatc

SEQ ID NO: 71 - DNA, 34 bp, Artificial Sequence
  primer FcY93A/N208Sss
gctgaatggcaaggaggccaagtgcaaggtctcc

SEQ ID NO: 72 - DNA, 34 bp, Artificial Sequence
  primer FcY93A/N208Sas
ggagaccttgcacttggcctccttgccattcagc

SEQ ID NO: 73 - protein, 221 aa, Artificial Sequence
  HMC001 Fc fragment
PSCPAPEFLGGPSVFLFPPKPKDTLMISRTPEVTCVVVDVSQEDPEVQFNWYVDGVEVHNAKTKPREEQFNSTYRVVSVLTVLHQDWLNGKEYKCKVSNKGLPSSIEKTISKAKGQPREPQVYTLPPSQEEMTKNQVSLTCLVKGFYPSDIAVEWESNGQPENNYKTTPPVLDSDGSFFLYSRLTVDKSRWQEGNVFSCSVMHEALHNHYTQKSLSLSLGK

SEQ ID NO: 74 - protein, 221 aa, Artificial Sequence
  HMC002 Fc fragment derivative
PSCPAPEFLGGPSVFLFPPKPKDTLMISRTPEVTCVVVDVSQEDPEVQFNWYVDGVEVHNAKTKPREEQFNSTYRVVSVLTVLHQDWLNGKEYKCKVSNKGLPSSIEKTISKAKGQPREPQVYTLPPSQEEMTKNQVSLTCLVKGFYPSDIAVEWESNGQPENNYKTTPPVLDSDGSFFLYSRLTVDKSRWQEGNVFSCSVLHEALHSHYTQKSLSLSLGK

SEQ ID NO: 75 - protein, 221 aa, Artificial Sequence
  HMC003 Fc fragment derivative
PSCPAPEFLGGPSVFLFPPKPKDTLMFSRTPEVTCVVVDVSQEDPEVQFNWYVDGVEVHNAKTKPREEQFNSTYRVVSVLTVLHQDWLNGKEYKCKVSNKGLPSSIEKTISKAKGQPREPQVYTLPPSQEEMTKNQVSLTCLVKGFYPSDIAVEWESNGQPENNYKTTPPVLDSDGSFFLYSRLTVDKSRWQEGNVFSCSVMHEALHNHYTQKSLSLSLGK

SEQ ID NO: 76 - protein, 221 aa, Artificial Sequence
  HMC004 Fc fragment derivative
PSCPAPEFLGGPSVFLFPPKPKDTLMISRTPEVTCVVVDVSQEDPEVQFNWYVDGVEVHNAKTKPREEQFNSTYRVVSVLTVLHQDWLNGKEYKCKVSNKGLPSSIEKTISKAKGQPREPQVYTLPPSQEEMTKNQVSLTCLVKGFYPSDIAVEWESNGQPENNYKTTPPVLDSDGSFFLYSRLTVDKSRWQEGNVFSCSVMHEALTNHYTQKSLSLSLGK

SEQ ID NO: 77 - protein, 221 aa, Artificial Sequence
  HMC005 Fc fragment derivative
PSCPAPEFLGGPSVFLFPPKPKDTLMISRTPEVTCVVVDVSQEDPEVQFNWYVDGVEVHNAKTKPREEQFNSTYRVVSVLTVLHQDWLNGKEYKCKVSNKGLPSSIEKTISKAKGQPREPQVYTLPPSQEEMTKNQVSLTCLVKGFYPSDIAVEWESNGQPENNYKTTPPVLDSDGSFFLYSRLTVDKSRWQEGNVFSCSVMHEALKNHYTQKSLSLSLGK

SEQ ID NO: 78 - protein, 221 aa, Artificial Sequence
  HMC006 Fc fragment derivative
PSCPAPEFLGGPSVFLFPPKPKDTLMISRTPEVTCVVVDVSQEDPEVQFNWYVDGVEVHNAKTKPREEQFNSTYRVVSVLTVFHQDWLNGKEYKCKVSNKGLPSSIEKTISKAKGQPREPQVYTLPPSQEEMTKNQVSLTCLVKGFYPSDIAVEWESNGQPENNYKTTPPVLDSDGSFFLYSRLTVDKSRWQEGNVFSCSVMHEALHSHYTQKSLSLSLGK

SEQ ID NO: 79 - protein, 221 aa, Artificial Sequence
  HMC007 Fc fragment derivative
PSCPAPEFLGGPSVFLFPPKPKDTLMLSRTPEVTCVVVDVSQEDPEVQFNWYVDGVEVHNAKTKPREEQFNSTYRVVSVLTVLHQDWLNGKEYKCKVSNKGLPSSIEKTISKAKGQPREPQVYTLPPSQEEMTKNQVSLTCLVKGFYPSDIAVEWESNGQPENNYKTTPPVLDSDGSFFLYSRLTVDKSRWQEGNVFSCSVMHEALHNHYTQKSLSLSLGK

SEQ ID NO: 80 - protein, 221 aa, Artificial Sequence
  HMC008 Fc fragment derivative
PSCPAPEFLGGPSVFLFPPKPKDTLMISRTPEVTCVVVDVSQEDPEVQFNWYVDGVEVHNAKTKPREEQFNSTYRVVSVLTVLHQDWLNGKEYKCKVSNKGLPSSIEKTISKAKGQPREPQVYTLPPSQEEMTKNQVSLTCLVKGFYPSDIAVEWESNGQPENNYKTTPPVLDSDGSFFLYSRLTVDKSRWQEGNVFSCSVMHEALKSHYTQKSLSLSLGK

SEQ ID NO: 81 - protein, 221 aa, Artificial Sequence
  HMC009 Fc fragment derivative
PSCPAPEFLGGPSVFLFPPKPKDTLMISRTPEVTCVVVDVSQEDPEVQFNWYVDGVEVHNAKTKPREEQFNSTYRVVSVLTVLHQDWLNGKEYKCKVSNKGLPSSIEKTISKAKGQPREPQVYTLPPSQEEMTKNQVSLTCLVKGFYPSDIAVEWESNGQPENNYKTTPPVLDSDGSFFLYSRLTVDKSRWQEGNVFSCSVMHEALHTHYTQKSLSLSLGK

SEQ ID NO: 82 - protein, 221 aa, Artificial Sequence
  HMC010 Fc fragment derivative
PSCPAPEFLGGPSVFLFPPKPKDTLMISRTPEVTCVVVDVSQEDPEVQFNWYVDGVEVHNAKTKPREEQFNSTYRVVSVLTVLHQDWLNGKEYKCKVSNKGLPSSIEKTISKAKGQPREPQVYTLPPSQEEMTKNQVSLTCLVKGFYPSDIAVEWESNGQPENNYKTTPPVLDSDGSFFLYSRLTVDKSRWQEGNVFSCSVMHEALTSHYTQKSLSLSLGK

SEQ ID NO: 83 - protein, 221 aa, Artificial Sequence
  HMC011 Fc fragment derivative
PSCPAPEFLGGPSVFLFPPKPKDTLMISRTPEVTCVVVDVSQEDPEVQFNWYVDGVEVHNAKTKPREEQFNSTYRVVSVLTVFHQDWLNGKEYKCKVSNKGLPSSIEKTISKAKGQPREPQVYTLPPSQEEMTKNQVSLTCLVKGFYPSDIAVEWESNGQPENNYKTTPPVLDSDGSFFLYSRLTVDKSRWQEGNVFSCSVMHEALHNHYTQKSLSLSLGK

SEQ ID NO: 84 - protein, 221 aa, Artificial Sequence
  HMC012 Fc fragment derivative
PSCPAPEFLGGPSVFLFPPKPKDTLMISRTPEVTCVVVDVSQEDPEVQFNWYVDGVEVHNAKTKPREEQFNSTYRVVSVLTVLHQDWLNGKEYKCKVSNKGLPSSIEKTISKAKGQPREPQVYTLPPSQEEMTKNQVSLTCLVKGFYPSDIAVEWESNGQPENNYKTTPPVLDSDGSFFLYSRLTVDKSRWQEGNVFSCSVMHRALHNHYTQKSLSLSLGK

SEQ ID NO: 85 - protein, 221 aa, Artificial Sequence
  HMC013 Fc fragment derivative
PSCPAPEFLGGPSVFLFPPKPKDTLMISRTPEVTCVVVDVSQEDPEVQFNWYVDGVEVHNAKTKPREEQFNSTYRVVSVLTVLHQDWLNGKEYKCKVSNKGLPSSIEKTISKAKGQPREPQVYTLPPSQEEMTKNQVSLTCLVKGFYPSDIAVEWESNGQPENNYKTTPPVLDSDGSFFLYSRLTVDKSRWQEGNVFSCSVMHKALHNHYTQKSLSLSLGK

SEQ ID NO: 86 - protein, 221 aa, Artificial Sequence
  HMC014 Fc fragment derivative
PSCPAPEFLGGPSVFLFPPKPKDTLMISRTPEVTCVVVDVSQEDPEVQFNWYVDGVEVHNAKTKPREEQFNSTYRVVSVLTVLHQDWLNGKEYKCKVSNKGLPSSIEKTISKAKGQPREPQVYTLPPSQEEMTKNQVSLTCLVKGFYPSDIAVEWESNGQPENNYKTTPPVLDSDGSFFLYSRLTVDKSRWQEGNVFSCSVMHRALKNHYTQKSLSLSLGK

SEQ ID NO: 87 - protein, 221 aa, Artificial Sequence
  HMC015 Fc fragment derivative
PSCPAPEFLGGPSVFLFPPKPKDTLMISRTPEVTCVVVDVSQEDPEVQFNWYVDGVEVHNAKTKPREEQFNSTYRVVSVLTVLHQDWLNGKEYKCKVSNKGLPSSIEKTISKAKGQPREPQVYTLPPSQEEMTKNQVSLTCLVKGFYPSDIAVEWESNGQPENNYKTTPPVLDSDGSFFLYSRLTVDKSRWQEGNVFSCSVMHKALKNHYTQKSLSLSLGK

SEQ ID NO: 88 - protein, 221 aa, Artificial Sequence
  HMC016 Fc fragment derivative
PSCPAPEFLGGPSVFLFPPKPKDTLMISRTPEVTCVVVDVSQEDPEVQFNWYVDGVEVHNAKTKPREEQFNSTYRVVSVLTVLHQDWLNGKEYKCKVSNKGLPSSIEKTISKAKGQPREPQVYTLPPSQEEMTKNQVSLTCLVKGFYPSDIAVEWESNGQPENNYKTTPPVLDSDGSFFLYSRLTVDKSRWQEGNVFSCSVMREALHNHYTQKSLSLSLGK

SEQ ID NO: 89 - protein, 221 aa, Artificial Sequence
  HMC017 Fc fragment derivative
PSCPAPEFLGGPSVFLFPPKPKDTLMISRTPEVTCVVVDVSQEDPEVQFNWYVDGVEVHNAKTKPREEQFNSTYRVVSVLTVLHQDWLNGKEYKCKVSNKGLPSSIEKTISKAKGQPREPQVYTLPPSQEEMTKNQVSLTCLVKGFYPSDIAVEWESNGQPENNYKTTPPVLDSDGSFFLYSRLTVDKSRWQEGNVFSCSVMKEALHNHYTQKSLSLSLGK

SEQ ID NO: 90 - protein, 221 aa, Artificial Sequence
  HMC018 Fc fragment derivative
PSCPAPEFLGGPSVFLFPPKPKDTLMISRTPEVTCVVVDVSQEDPEVQFNWYVDGVEVHNAKTKPREEQFNSTYRVVSVLTVLHQDWLNGKEYKCKVSNKGLPSSIEKTISKAKGQPREPQVYTLPPSQEEMTKNQVSLTCLVKGFYPSDIAVEWESNGQPENNYKTTPPVLDSDGSFFLYSRLTVDKSRWQEGNVFSCSVMREALKNHYTQKSLSLSLGK

SEQ ID NO: 91 - protein, 221 aa, Artificial Sequence
  HMC019 Fc fragment derivative
PSCPAPEFLGGPSVFLFPPKPKDTLMISRTPEVTCVVVDVSQEDPEVQFNWYVDGVEVHNAKTKPREEQFNSTYRVVSVLTVLHQDWLNGKEYKCKVSNKGLPSSIEKTISKAKGQPREPQVYTLPPSQEEMTKNQVSLTCLVKGFYPSDIAVEWESNGQPENNYKTTPPVLDSDGSFFLYSRLTVDKSRWQEGNVFSCSVMKEALKNHYTQKSLSLSLGK

SEQ ID NO: 92 - protein, 221 aa, Artificial Sequence
  HMC020 Fc fragment derivative
PSCPAPEFLGGPSVFLFPPKPKDTLMISRTPEVTCVVVDVSQEDPEVQFNWYVDGVEVHNAKTKPREEQFNSTYRVVSVLTVLHQDWLNGKEYKCKVSNKGLPSSIEKTISKAKGQPREPQVYTLPPSQEEMTKNQVSLTCLVKGFYPSDIAVEWESNGQPENNYKTTPPVLDSDGSFFLYSRLTVDKSRWQEGNVFSCSVLHEALKNHYTQKSLSLSLGK

SEQ ID NO: 93 - protein, 221 aa, Artificial Sequence
  HMC021 Fc fragment derivative
PSCPAPEFLGGPSVFLFPPKPKDTLMISRTPEVTCVVVDVSQEDPEVQFNWYVDGVEVHNAKTKPREEQFNSTYRVVSVLTVLHQDWLNGKEYKCKVSNKGLPSSIEKTISKAKGQPREPQVYTLPPSQEEMTKNQVSLTCLVKGFYPSDIAVEWESNGQPENNYKTTPPVLDSDGSFFLYSRLTVDKSRWQEGNVFSCSVMKEALHTHYTQKSLSLSLGK

SEQ ID NO: 94 - protein, 221 aa, Artificial Sequence
  HMC022 Fc fragment derivative
PSCPAPEFLGGPSVFLFPPKPKDTLMISRTPEVTCVVVDVSQEDPEVQFNWYVDGVEVHNAKTKPREEQFNSTYRVVSVLEVLHQDWLNGKEYKCKVSNKGLPSSIEKTISKAKGQPREPQVYTLPPSQEEMTKNQVSLTCLVKGFYPSDIAVEWESNGQPENNYKTTPPVLDSDGSFFLYSRLTVDKSRWQEGNVFSCSVMHEALHNHYTQKSLSLSLGK

SEQ ID NO: 95 - protein, 221 aa, Artificial Sequence
  HMC023 Fc fragment derivative
PSCPAPEFLGGPSVFLFPPKPKDTLMISRTPEVTCVVVDVSQEDPEVQFNWYVDGVEVHNAKTKPREEQFNSTYRVVSVLEVLHQDWLNGKEYKCKVSNKGLPSSIEKTISKAKGQPREPQVYTLPPSQEEMTKNQVSLTCLVKGFYPSDIAVEWESNGQPENNYKTTPPVLDSDGSFFLYSRLTVDKSRWQEGNVFSCSVLHEALHNHYTQKSLSLSLGK

SEQ ID NO: 96 - protein, 221 aa, Artificial Sequence
  HMC024 Fc fragment derivative
PSCPAPEFLGGPSVFLFPPKPKDTLMISRTPEVTCVVVDVSQEDPEVQFNWYVDGVEVHNAKTKPREEQFNSTYRVVSVLTVLHQDWLNGKEYKCKVSNKGLPSSIEKTISKAKGQPREPQVYTLPPSQEEMTKNQVSLTCLVKGFYPSDIAVAWESNGQPENNYKTTPPVLDSDGSFFLYSRLTVDKSRWQEGNVFSCSVMHEALHNHYTQKSLSLSLGK

SEQ ID NO: 97 - protein, 221 aa, Artificial Sequence
  HMC025 Fc fragment derivative
PSCPAPEFLGGPSVFLFPPKPKDTLMISRTPEVTCVVVDVSQEDPEVQFNWYVDGVEVHNAKTKPREEQFNSTYRVVSVLTVLHQDWLNGKEYKCKVSNKGLPSSIEKTISKAKGQPREPQVYTLPPSQEEMTKNQVSLTCLVKGFYPSDIAVSWESNGQPENNYKTTPPVLDSDGSFFLYSRLTVDKSRWQEGNVFSCSVMHEALHNHYTQKSLSLSLGK

SEQ ID NO: 98 - protein, 221 aa, Artificial Sequence
  HMC026 Fc fragment derivative
PSCPAPEFLGGPSVFLFPPKPKDTLMISRTPEVTCVVVDVSQEDPEVQFNWYVDGVEVHNAKTKPREEQFNSTYRVVSVLTVLHQDWLNGKEYKCKVSNKGLPSSIEKTISKAKGQPREPQVYTLPPSQEEMTKNQVSLTCLVKGFYPSDIAVAWESNGQPENNYKTTPPVLDSDGSFFLYSRLTVDKSRWQEGNVFSCSVMHEALHSHYTQKSLSLSLGK

SEQ ID NO: 99 - protein, 221 aa, Artificial Sequence
  HMC027 Fc fragment derivative
PSCPAPEFLGGPSVFLFPPKPKDTLMISRTPEVTCVVVDVSQEDPEVQFNWYVDGVEVHNAKTKPREEQFNSTYRVVSVLTFLHQDWLNGKEYKCKVSNKGLPSSIEKTISKAKGQPREPQVYTLPPSQEEMTKNQVSLTCLVKGFYPSDIAVEWESNGQPENNYKTTPPVLDSDGSFFLYSRLTVDKSRWQEGNVFSCSVMHSALHSHYTQKSLSLSLGK

SEQ ID NO: 100 - protein, 221 aa, Artificial Sequence
  HMC028 Fc fragment derivative
PSCPAPEFLGGPSVFLFPPKPKDTLMISRTPEVTCVVVDVSQEDPEVQFNWYVDGVEVHNAKTKPREEQFNSTYRVVSVLTFLHQDWLNGKEYKCKVSNKGLPSSIEKTISKAKGQPREPQVYTLPPSQEEMTKNQVSLTCLVKGFYPSDIAVAWESNGQPENNYKTTPPVLDSDGSFFLYSRLTVDKSRWQEGNVFSCSVMHEALHNHYTQKSLSLSLGK

SEQ ID NO: 101 - protein, 221 aa, Artificial Sequence
  HMC029 Fc fragment derivative
PSCPAPEFLGGPSVFLFPPKPKDTLMISRTPEVTCVVVDVSQEDPEVQFNWYVDGVEVHNAKTKPREEQFNSTYRVVSVLSVLHQDWLNGKEYKCKVSNKGLPSSIEKTISKAKGQPREPQVYTLPPSQEEMTKNQVSLTCLVKGFYPSDIAVSWESNGQPENNYKTTPPVLDSDGSFFLYSRLTVDKSRWQEGNVFSCSVMHEALHNHYTQKSLSLSLGK

SEQ ID NO: 102 - protein, 221 aa, Artificial Sequence
  HMC030 Fc fragment derivative
PSCPAPEFLGGPSVFLFPPKPKDTLMISRTPEVTCVVVDVSQEDPEVQFNWYVDGVEVHNAKTKPREEQFNSTYRVVSVLTVLHQDWLNGKEYKCKVSNKGLPSSIEKTISKAKGQPREPQVYTLPPSQEEMTKNQVSLTCLVKGFYPSDIAVEWESNGQPENNYKTTPPVLDSDGSFFLYSRLTVDKSRWQEGNVFSCSVMASALHNHYTQKSLSLSLGK

SEQ ID NO: 103 - protein, 221 aa, Artificial Sequence
  HMC031 Fc fragment derivative
PSCPAPEFLGGPSVFLFPPKPKDTLMISRTPEVTCVVVDVSQEDPEVQFNWYVDGVEVHNAKTKPREEQFNSTYRVVSVLTVLHQDWLNGKEYKCKVSNKGLPSSIEKTISKAKGQPREPQVYTLPPSQEEMTKNQVSLTCLVKGFYPSDIAVSWESNGQPENNYKTTPPVLDSDGSFFLYSRLTVDKSRWQEGNVFSCSVMHEALHSHYTQKSLSLSLGK

SEQ ID NO: 104 - protein, 221 aa, Artificial Sequence
  HMC032 Fc fragment derivative
PSCPAPEFLGGPSVFLFPPKPKDTLMISRTPEVTCVVVDVSQEDPEVQFNWYVDGVEVHNAKTKPREEQFNSTYRVVSVLTVLHQDWLNGKEYKCKVSNKGLPSSIEKTISKAKGQPREPQVYTLPPSQEEMTKNQVSLTCLVKGFYPSDIAVEWESNGQPENNYKTTPPVLDSDGSFFLYSRLTVDKSRWQEGNVFSCSVMHEALASHYTQKSLSLSLGK

SEQ ID NO: 105 - protein, 221 aa, Artificial Sequence
  HMC033 Fc fragment derivative
PSCPAPEFLGGPSVFLFPPKPKDTLMISRTPEVTCVVVDVSQEDPEVQFNWYVDGVEVHNAKTKPREEQFNSTYRVVSVLTVLHQDWLNGKEYKCKVSNKGLPSSIEKTISKAKGQPREPQVYTLPPSQEEMTKNQVSLTCLVKGFYPSDIAVEWESNGQPENNYKTTPPVLDSDGSFFLYSRLTVDKSRWQEGNVFSCSVMHAALHSHYTQKSLSLSLGK

SEQ ID NO: 106 - protein, 221 aa, Artificial Sequence
  HMC034 Fc fragment derivative
PSCPAPEFLGGPSVFLFPPKPKDTLMISRTPEVTCVVVDVSQEDPEVQFNWYVDGVEVHNAKTKPREEQFNSTYRVVSVLTVLHQDWLNGKEYKCKVSNKGLPSSIEKTISKAKGQPREPQVYTLPPSQEEMTKNQVSLTCLVKGFYPSDIAVEWESNGQPENNYKTTPPVLDSDGSFFLYSRLTVDKSRWQEGNVFSCSVMAEALHSHYTQKSLSLSLGK

SEQ ID NO: 107 - protein, 221 aa, Artificial Sequence
  HMC035 Fc fragment derivative
PSCPAPEFLGGPSVFLFPPKPKDTLMISRTPEVTCVVVDVSQEDPEVQFNWYVDGVEVHNAKTKPREEQFNSTYRVVSVLTVLHQDWLNGKEYKCKVSNKGLPSSIEKTISKAKGQPREPQVYTLPPSQEEMTKNQVSLTCLVKGFYPSDIAVEWESNGQPENNYKTTPPVLDSDGSFFLYSRLTVDKSRWQEGNVFSCSVAHEALHSHYTQKSLSLSLGK

SEQ ID NO: 108 - protein, 221 aa, Artificial Sequence
  HMC036 Fc fragment derivative
PSCPAPEFLGGPSVFLFPPKPKDTLMISRTPEVTCVVVDVSQEDPEVQFNWYVDGVEVHNAKTKPREEQFNSTYRVVSVLTVLHQDWLNGKELKCKVSNKGLPSSIEKTISKAKGQPREPQVYTLPPSQEEMTKNQVSLTCLVKGFYPSDIAVEWESNGQPENNYKTTPPVLDSDGSFFLYSRLTVDKSRWQEGNVFSCSVMHEALHSHYTQKSLSLSLGK

SEQ ID NO: 109 - protein, 221 aa, Artificial Sequence
  HMC037 Fc fragment derivative
PSCPAPEFLGGPSVFLFPPKPKDTLMISRTPEVTCVVVDVSQEDPEVQFNWYVDGVEVHNAKTKPREEQFNSTYRVVSVLTLLHQDWLNGKEYKCKVSNKGLPSSIEKTISKAKGQPREPQVYTLPPSQEEMTKNQVSLTCLVKGFYPSDIAVEWESNGQPENNYKTTPPVLDSDGSFFLYSRLTVDKSRWQEGNVFSCSVMHEALHSHYTQKSLSLSLGK

SEQ ID NO: 110 - protein, 221 aa, Artificial Sequence
  HMC038 Fc fragment derivative
PSCPAPEFLGGPSVFLFPPKPKDTLMISRTPEVTCVVVDVSQEDPEVQFNWYVDGVEVHNAKTKPREEQFNSTYRVVSVLAVLHQDWLNGKEYKCKVSNKGLPSSIEKTISKAKGQPREPQVYTLPPSQEEMTKNQVSLTCLVKGFYPSDIAVEWESNGQPENNYKTTPPVLDSDGSFFLYSRLTVDKSRWQEGNVFSCSVMHEALHSHYTQKSLSLSLGK

SEQ ID NO: 111 - protein, 221 aa, Artificial Sequence
  HMC039 Fc fragment derivative
PSCPAPEFLGGPSVFLFPPKPKDTLMISRTPEVTCVVVDVSQEDPEVQFNWYVDGVEVHNAKTKPREEQFNSTYRVVSVLTVLHQDWLNGKEYKCKVSNKGLPSSIEKTISKAKGQPREPQVYTLPPSQEEMTKNQVSLTCLVKGFYPSDIAVEWESNGQPENNYKTTPPVLDSDGSFFLYSRLTVDKSRWQEGNVFSCSVMHEALLSHYTQKSLSLSLGK

SEQ ID NO: 112 - protein, 221 aa, Artificial Sequence
  HMC040 Fc fragment derivative
PSCPAPEFLGGPSVFLFPPKPKDTLMISRTPEVTCVVVDVSQEDPEVQFNWYVDGVEVHNAKTKPREEQFNSTYRVVSVLTVLHQDWLNGKEAKCKVSNKGLPSSIEKTISKAKGQPREPQVYTLPPSQEEMTKNQVSLTCLVKGFYPSDIAVEWESNGQPENNYKTTPPVLDSDGSFFLYSRLTVDKSRWQEGNVFSCSVMHEALHSHYTQKSLSLSLGK

SEQ ID NO: 113 - DNA, 663 bp, Artificial Sequence
  HMC002 Fc fragment derivative
ccatcatgcccagcacctgagttcctggggggaccatcagtcttcctgttccccccaaaacccaaggacaccctcatgatctcccggacccctgaggtcacatgcgtggtggtggacgtgagccaggaagaccctgaggtccagttcaactggtacgtggacggcgtggaggtgcataatgccaagacaaagccgcgggaggagcagttcaacagcacgtaccgtgtggtcagcgtcctcaccgtcctgcaccaggactggctgaatggcaaggagtacaagtgcaaggtctccaacaaaggcctcccatcctccatcgagaaaaccatctccaaagccaaagggcagccccgagaaccacaggtgtacaccctgcccccatcccaggaggagatgaccaagaaccaggtcagcctgacctgcctggtcaaaggcttctatcccagcgacatcgccgtggagtgggagagcaatgggcagccggagaacaactacaagaccacgcctcccgtgctggactccgacggctccttcttcctctacagcaggctaaccgtggacaagagcaggtggcaggaggggaacgtcttctcatgctccgtgctgcatgaggctctgcacagccactacacacagaagagcctctccctgtctctgggtaaa

SEQ ID NO: 114 - DNA, 663 bp, Artificial Sequence
  HMC008 Fc fragment derivative
ccatcatgcccagcacctgagttcctggggggaccatcagtcttcctgttccccccaaaacccaaggacaccctcatgatctcccggacccctgaggtcacatgcgtggtggtggacgtgagccaggaagaccctgaggtccagttcaactggtacgtggacggcgtggaggtgcataatgccaagacaaagccgcgggaggagcagttcaacagcacgtaccgtgtggtcagcgtcctcaccgtcctgcaccaggactggctgaatggcaaggagtacaagtgcaaggtctccaacaaaggcctcccatcctccatcgagaaaaccatctccaaagccaaagggcagccccgagaaccacaggtgtacaccctgcccccatcccaggaggagatgaccaagaaccaggtcagcctgacctgcctggtcaaaggcttctatcccagcgacatcgccgtggagtgggagagcaatgggcagccggagaacaactacaagaccacgcctcccgtgctggactccgacggctccttcttcctctacagcaggctaaccgtggacaagagcaggtggcaggaggggaacgtcttctcatgctccgtgatgcatgaggctctgaagagccactacacacagaagagcctctccctgtctctgggtaaa

SEQ ID NO: 115 - DNA, 663 bp, Artificial Sequence
  HMC019 Fc fragment derivative
ccatcatgcccagcacctgagttcctggggggaccatcagtcttcctgttccccccaaaacccaaggacaccctcatgatctcccggacccctgaggtcacatgcgtggtggtggacgtgagccaggaagaccctgaggtccagttcaactggtacgtggacggcgtggaggtgcataatgccaagacaaagccgcgggaggagcagttcaacagcacgtaccgtgtggtcagcgtcctcaccgtcctgcaccaggactggctgaatggcaaggagtacaagtgcaaggtctccaacaaaggcctcccatcctccatcgagaaaaccatctccaaagccaaagggcagccccgagaaccacaggtgtacaccctgcccccatcccaggaggagatgaccaagaaccaggtcagcctgacctgcctggtcaaaggcttctatcccagcgacatcgccgtggagtgggagagcaatgggcagccggagaacaactacaagaccacgcctcccgtgctggactccgacggctccttcttcctctacagcaggctaaccgtggacaagagcaggtggcaggaggggaacgtcttctcatgctccgtgatgaaggaggctctgaagaaccactacacacagaagagcctctccctgtctctgggtaaa

SEQ ID NO: 116 - DNA, 663 bp, Artificial Sequence
  HMC020 Fc fragment derivative
ccatcatgcccagcacctgagttcctggggggaccatcagtcttcctgttccccccaaaacccaaggacaccctcatgatctcccggacccctgaggtcacatgcgtggtggtggacgtgagccaggaagaccctgaggtccagttcaactggtacgtggacggcgtggaggtgcataatgccaagacaaagccgcgggaggagcagttcaacagcacgtaccgtgtggtcagcgtcctcaccgtcctgcaccaggactggctgaatggcaaggagtacaagtgcaaggtctccaacaaaggcctcccatcctccatcgagaaaaccatctccaaagccaaagggcagccccgagaaccacaggtgtacaccctgcccccatcccaggaggagatgaccaagaaccaggtcagcctgacctgcctggtcaaaggcttctatcccagcgacatcgccgtggagtgggagagcaatgggcagccggagaacaactacaagaccacgcctcccgtgctggactccgacggctccttcttcctctacagcaggctaaccgtggacaagagcaggtggcaggaggggaacgtcttctcatgctccgtgctgcatgaggctctgaagaaccactacacacagaagagcctctccctgtctctgggtaaa

SEQ ID NO: 117 - DNA, 663 bp, Artificial Sequence
  HMC028 Fc fragment derivative
ccatcatgcccagcacctgagttcctggggggaccatcagtcttcctgttccccccaaaacccaaggacaccctcatgatctcccggacccctgaggtcacatgcgtggtggtggacgtgagccaggaagaccctgaggtccagttcaactggtacgtggacggcgtggaggtgcataatgccaagacaaagccgcgggaggagcagttcaacagcacgtaccgtgtggtcagcgtcctcacccccctgcaccaggactggctgaatggcaaggagtacaagtgcaaggtctccaacaaaggcctcccatcctccatcgagaaaaccatctccaaagccaaagggcagccccgagaaccacaggtgtacaccctgcccccatcccaggaggagatgaccaagaaccaggtcagcctgacctgcctggtcaaaggcttctatcccagcgacatcgccgtggcgtgggagagcaatgggcagccggagaacaactacaagaccacgcctcccgtgctggactccgacggctccttcttcctctacagcaggctaaccgtggacaagagcaggtggcaggaggggaacgtcttctcatgctccgtgatgcatgaggctctgcacaaccactacacacagaagagcctctccctgtctctgggtaaa

SEQ ID NO: 118 - DNA, 663 bp, Artificial Sequence
  HMC029 Fc fragment derivative
ccatcatgcccagcacctgagttcctggggggaccatcagtcttcctgttccccccaaaacccaaggacaccctcatgatctcccggacccctgaggtcacatgcgtggtggtggacgtgagccaggaagaccctgaggtccagttcaactggtacgtggacggcgtggaggtgcataatgccaagacaaagccgcgggaggagcagttcaacagcacgtaccgtgtggtcagcgtcctctccgtcctgcaccaggactggctgaatggcaaggagtacaagtgcaaggtctccaacaaaggcctcccatcctccatcgagaaaaccatctccaaagccaaagggcagccccgagaaccacaggtgtacaccctgcccccatcccaggaggagatgaccaagaaccaggtcagcctgacctgcctggtcaaaggcttctatcccagcgacatcgccgtgtcgtgggagagcaatgggcagccggagaacaactacaagaccacgcctcccgtgctggactccgacggctccttcttcctctacagcaggctaaccgtggacaagagcaggtggcaggaggggaacgtcttctcatgctccgtgatgcatgaggctctgcacaaccactacacacagaagagcctctccctgtctctgggtaaa

SEQ ID NO: 119 - DNA, 663 bp, Artificial Sequence
  HMC031 Fc fragment derivative
ccatcatgcccagcacctgagttcctggggggaccatcagtcttcctgttccccccaaaacccaaggacaccctcatgatctcccggacccctgaggtcacatgcgtggtggtggacgtgagccaggaagaccctgaggtccagttcaactggtacgtggacggcgtggaggtgcataatgccaagacaaagccgcgggaggagcagttcaacagcacgtaccgtgtggtcagcgtcctcaccgtcctgcaccaggactggctgaatggcaaggagtacaagtgcaaggtctccaacaaaggcctcccatcctccatcgagaaaaccatctccaaagccaaagggcagccccgagaaccacaggtgtacaccctgcccccatcccaggaggagatgaccaagaaccaggtcagcctgacctgcctggtcaaaggcttctatcccagcgacatcgccgtgtcgtgggagagcaatgggcagccggagaacaactacaagaccacgcctcccgtgctggactccgacggctccttcttcctctacagcaggctaaccgtggacaagagcaggtggcaggaggggaacgtcttctcatgctccgtgatgcatgaggctctgcacagccactacacacagaagagcctctccctgtctctgggtaaa